European Patent Application EP 4 170 043 A1, published April 26, 2023. Title: Fetal Genomic Analysis from a Maternal Biological Sample. Applicant: The Chinese University Of Hong Kong. Application EP, filed November 5, 2010. The sequence listing filed with the application follows.

SEQUENCE LISTING (52 sequences)

SEQ ID NO: 1 - DNA, 14 bp, synthetic construct
  misc_feature 1..14: note = synthetic haplotype A (Hap A)
  source 1..14: mol_type = other DNA
acgatacgattaag

SEQ ID NO: 2 - DNA, 14 bp, synthetic construct
  misc_feature 1..14: note = synthetic haplotype B (Hap B)
  source 1..14: mol_type = other DNA
cggtagccttatcg

SEQ ID NO: 3 - DNA, 14 bp, synthetic construct
  misc_feature 1..14: note = synthetic haplotype C (Hap C)
  source 1..14: mol_type = other DNA
ccattgtcagttca

SEQ ID NO: 4 - DNA, 14 bp, synthetic construct
  misc_feature 1..14: note = synthetic maternal genotypes
  source 1..14: mol_type = other DNA
msgwwrcswtwwmg

SEQ ID NO: 5 - DNA, 50 bp, Homo sapiens
  misc_feature 1..50: note = synthetic read with codons 41/42 paternally inherited mutation
  source 1..50: mol_type = other DNA
cgggtattgtcgtagtcctcacctgtctaggggtttcctgagttggagac

SEQ ID NO: 6 - DNA, 50 bp, Homo sapiens
  misc_feature 1..50: note = synthetic read with codons 41/42 paternally inherited mutation
  source 1..50: mol_type = other DNA
gggtattgtcgtagtcctcacctgtctaggggtttcctgagttggagacc

SEQ ID NO: 7 - DNA, 50 bp, Homo sapiens
  misc_feature 1..50: note = synthetic read with codons 41/42 paternally inherited mutation
  source 1..50: mol_type = other DNA
ggtattgtcgtagtcctcacctgtctaggggtttcctgagttggagaccc

SEQ ID NO: 8 - DNA, 50 bp, Homo sapiens
  misc_feature 1..50: note = synthetic read with codons 41/42 paternally inherited mutation
  source 1..50: mol_type = other DNA
cgtagtcctcacctgtctaggggtttcctgagttggagacccaggttccc

SEQ ID NO: 9 - DNA, 50 bp, Homo sapiens
  misc_feature 1..50: note = synthetic read with codons 41/42 paternally inherited mutation
  source 1..50: mol_type = other DNA
gtagtcctcacctgtctaggggtttcctgagttggagacccaggttccca

SEQ ID NO: 10 - DNA, 50 bp, Homo sapiens
  misc_feature 1..50: note = synthetic read with codons 41/42 paternally inherited mutation
  source 1..50: mol_type = other DNA
ctgtctaggggtttcctgagttggagacccaggttcccatctggtggtcg

SEQ ID NO: 11 - DNA, 50 bp, Homo sapiens
  misc_feature 1..50: note = synthetic read with codons 41/42 paternally inherited mutation
  source 1..50: mol_type = other DNA
tgtctaggggtttcctgagttggagacccaggttcccatctggtggtcgt

SEQ ID NO: 12 - DNA, 50 bp, Homo sapiens
  misc_feature 1..50: note = synthetic read with codons 41/42 paternally inherited mutation
  source 1..50: mol_type = other DNA
ttcctgagtgggagacccaggttcccatctggtggtcgtcggattcccac

SEQ ID NO: 13 - DNA, 50 bp, Homo sapiens
  misc_feature 1..50: note = synthetic read with codons 41/42 paternally inherited mutation
  source 1..50: mol_type = other DNA
gtgggagacccaggttcccatctggtggtcgtcggattcccaccctttta

SEQ ID NO: 14 - DNA, 44 bp, Homo sapiens
  misc_feature 1..44: note = synthetic read with codons 41/42 wildtype sequence
  source 1..44: mol_type = other DNA
gtattgtcgtagtcctcacctgtctaggggtttcctgagtttct

SEQ ID NO: 15 - DNA, 45 bp, Homo sapiens
  misc_feature 1..45: note = synthetic read with codons 41/42 wildtype sequence
  source 1..45: mol_type = other DNA
gtattgtcgtagtcctcacctgtctaggggtttcctgagtttctt

SEQ ID NO: 16 - DNA, 46 bp, Homo sapiens
  misc_feature 1..46: note = synthetic read with codons 41/42 wildtype sequence
  source 1..46: mol_type = other DNA
gtattgtcgtagtcctcacctgtctaggggtttcctgagtttcttg

SEQ ID NO: 17 - DNA, 47 bp, Homo sapiens
  misc_feature 1..47: note = synthetic read with codons 41/42 wildtype sequence
  source 1..47: mol_type = other DNA
gtattgtcgtagtcctcacctgtctaggggtttcctgagtttcttgg

SEQ ID NO: 18 - DNA, 47 bp, Homo sapiens
  misc_feature 1..47: note = synthetic read with codons 41/42 wildtype sequence
  source 1..47: mol_type = other DNA
gtatcgtcgtagtcctcacctgtctaggggtttcctgagtttcttgg

SEQ ID NO: 19 - DNA, 48 bp, Homo sapiens
  misc_feature 1..48: note = synthetic read with codons 41/42 wildtype sequence
  source 1..48: mol_type = other DNA
gtattgtcgtagtcctcacctgtctaggggtttcctgagtttcttgga

SEQ ID NO: 20 - DNA, 49 bp, Homo sapiens
  misc_feature 1..49: note = synthetic read with codons 41/42 wildtype sequence
  source 1..49: mol_type = other DNA
gtattgtcgtagtcctcacctgtctaggggtttcctgagtttcttggag

SEQ ID NO: 21 - DNA, 50 bp, Homo sapiens
  misc_feature 1..50: note = synthetic read with codons 41/42 wildtype sequence
  source 1..50: mol_type = other DNA
tattgtcgtagtcctcacctgtctaggggtttcctgagtttcttggagac

SEQ ID NO: 22 - DNA, 50 bp, Homo sapiens
  misc_feature 1..50: note = synthetic read with codons 41/42 wildtype sequence
  source 1..50: mol_type = other DNA
attgtcgtagtcctcacctgtctaggggtttcctgagtttcttggagacc

SEQ ID NO: 23 - DNA, 50 bp, Homo sapiens
  misc_feature 1..50: note = synthetic read with codons 41/42 wildtype sequence
  source 1..50: mol_type = other DNA
ttgtcgtagtcctcacctgtctaggggtttcctgagtttcttggagaccc

SEQ ID NO: 24 - DNA, 50 bp, Homo sapiens
  misc_feature 1..50: note = synthetic read with codons 41/42 wildtype sequence
  source 1..50: mol_type = other DNA
tcgtagtcctcacctgtctaggggtttcctgagtttcttggagacccagg

SEQ ID NO: 25 - DNA, 50 bp, Homo sapiens
  misc_feature 1..50: note = synthetic read with codons 41/42 wildtype sequence
  source 1..50: mol_type = other DNA
tcggagtcctcacctgtctaggggtttcctgagtttcttggagacccagg

SEQ ID NO: 26 - DNA, 50 bp, Homo sapiens
  misc_feature 1..50: note = synthetic read with codons 41/42 wildtype sequence
  source 1..50: mol_type = other DNA
cgtagtcctcacctgtctaggggtttcctgagtttcttggagacccaggt

SEQ ID NO: 27 - DNA, 50 bp, Homo sapiens
  misc_feature 1..50: note = synthetic read with codons 41/42 wildtype sequence
  source 1..50: mol_type = other DNA
gtagtcctcacctgtctaggggtttcctgagtttcttggagacccaggtt

SEQ ID NO: 28 - DNA, 50 bp, Homo sapiens
  misc_feature 1..50: note = synthetic read with codons 41/42 wildtype sequence
  source 1..50: mol_type = other DNA
tagtcctcacctgtctaggggtttcctgagtttcttggagacccaggttc

SEQ ID NO: 29 - DNA, 50 bp, Homo sapiens
  misc_feature 1..50: note = synthetic read with codons 41/42 wildtype sequence
  source 1..50: mol_type = other DNA
agtcctcacctgtctaggggtttcctgagtttcttggagacccaggttcc

SEQ ID NO: 30 - DNA, 50 bp, Homo sapiens
  misc_feature 1..50: note = synthetic read with codons 41/42 wildtype sequence
  source 1..50: mol_type = other DNA
gtcctcacctgtctaggggtttcctgagtttcttggagacccaggttccc

SEQ ID NO: 31 - DNA, 50 bp, Homo sapiens
  misc_feature 1..50: note = synthetic read with codons 41/42 wildtype sequence
  source 1..50: mol_type = other DNA
gccctcacctgtctaggggtttcctgagtttcttggagacccaggttccc

SEQ ID NO: 32 - DNA, 50 bp, Homo sapiens
  misc_feature 1..50: note = synthetic read with codons 41/42 wildtype sequence
  source 1..50: mol_type = other DNA
cctcacctgtctaggggtttcctgagtttcttggagacccaggttcccat

SEQ ID NO: 33 - DNA, 50 bp, Homo sapiens
  misc_feature 1..50: note = synthetic read with codons 41/42 wildtype sequence
  source 1..50: mol_type = other DNA
tcacctgtctaggggtttcctgagtttcttggagacccaggttcccatct

SEQ ID NO: 34 - DNA, 50 bp, Homo sapiens
  misc_feature 1..50: note = synthetic read with codons 41/42 wildtype sequence
  source 1..50: mol_type = other DNA
acgtgtctaggggtttcctgagtttcttggagacccaggttcccatctgg

SEQ ID NO: 35 - DNA, 50 bp, Homo sapiens
  misc_feature 1..50: note = synthetic read with codons 41/42 wildtype sequence
  source 1..50: mol_type = other DNA
acctgtctaggggtttcctgagtttcttggagacccaggttcccatctgg

SEQ ID NO: 36 - DNA, 50 bp, Homo sapiens
  misc_feature 1..50: note = synthetic read with codons 41/42 wildtype sequence
  source 1..50: mol_type = other DNA
cctgtctaggggtttcctgagtttcttggagacccaggttcccatctggt

SEQ ID NO: 37 - DNA, 50 bp, Homo sapiens
  misc_feature 1..50: note = synthetic read with codons 41/42 wildtype sequence
  source 1..50: mol_type = other DNA
gtctaggggtttcctgagtttcttggagacccaggttcccatctggtggt

SEQ ID NO: 38 - DNA, 50 bp, Homo sapiens
  misc_feature 1..50: note = synthetic read with codons 41/42 wildtype sequence
  source 1..50: mol_type = other DNA
ctaggggtttcctgagtttcttggagacccaggttcccatctggtggtcg

SEQ ID NO: 39 - DNA, 50 bp, Homo sapiens
  misc_feature 1..50: note = synthetic read with codons 41/42 wildtype sequence
  source 1..50: mol_type = other DNA
aggggtttcctgagtttcttggagacccaggttcccatctggtggtcgtc

SEQ ID NO: 40 - DNA, 50 bp, Homo sapiens
  misc_feature 1..50: note = synthetic read with codons 41/42 wildtype sequence
  source 1..50: mol_type = other DNA
aggggtttcctgagtttctgggagacccaggttcccatctgggggtcgtc

SEQ ID NO: 41 - DNA, 50 bp, Homo sapiens
  misc_feature 1..50: note = synthetic read with codons 41/42 wildtype sequence
  source 1..50: mol_type = other DNA
ggggtttcctgagtttcttggagacccaggttcccatctggtggtcgtcg

SEQ ID NO: 42 - DNA, 50 bp, Homo sapiens
  misc_feature 1..50: note = synthetic read with codons 41/42 wildtype sequence
  source 1..50: mol_type = other DNA
gggtttcctgagtttcttggagacccaggttcccatctggtggtcgtcgg

SEQ ID NO: 43 - DNA, 50 bp, Homo sapiens
  misc_feature 1..50: note = synthetic read with codons 41/42 wildtype sequence
  source 1..50: mol_type = other DNA
ggtttcctgagtttcttggagacccaggttcccatctggtggtcgtcgga

SEQ ID NO: 44 - DNA, 50 bp, Homo sapiens
  misc_feature 1..50: note = synthetic read with codons 41/42 wildtype sequence
  source 1..50: mol_type = other DNA
gtttcctgattttcttggagacccagggtcccatctggtggtcgtcggat

SEQ ID NO: 45 - DNA, 50 bp, Homo sapiens
  misc_feature 1..50: note = synthetic read with codons 41/42 wildtype sequence
  source 1..50: mol_type = other DNA
gtttcctgagtttcttggagacccaggttcccatctggtggtcgtcggat

SEQ ID NO: 46 - DNA, 50 bp, Homo sapiens
  misc_feature 1..50: note = synthetic read with codons 41/42 wildtype sequence
  source 1..50: mol_type = other DNA
ttcctgagtttcttggagacccaggttcccatctggtggtcgtcggattc

SEQ ID NO: 47 - DNA, 50 bp, Homo sapiens
  misc_feature 1..50: note = synthetic read with codons 41/42 wildtype sequence
  source 1..50: mol_type = other DNA
cctgagtttcttggagacccaggttcccatctggtggtcgtcggattccc

SEQ ID NO: 48 - DNA, 50 bp, Homo sapiens
  misc_feature 1..50: note = synthetic read with codons 41/42 wildtype sequence
  source 1..50: mol_type = other DNA
tgagtttcttggagacccaggttcccatctggtggtcgtcggattcccac

SEQ ID NO: 49 - DNA, 50 bp, Homo sapiens
  misc_feature 1..50: note = synthetic read with codons 41/42 wildtype sequence
  source 1..50: mol_type = other DNA
tgagttccttggagacccaggttcccatctgggggtcgtcggattcccac

SEQ ID NO: 50 - DNA, 50 bp, Homo sapiens
  misc_feature 1..50: note = synthetic read with codons 41/42 wildtype sequence
  source 1..50: mol_type = other DNA
gatgtccttggagacccaggttcccatctgggggtcgtcggattcccacc

SEQ ID NO: 51 - DNA, 50 bp, Homo sapiens
  misc_feature 1..50: note = synthetic read with codons 41/42 wildtype sequence
  source 1..50: mol_type = other DNA
gagtttgttggagacccaggttcccatctgggggtcgtcggattcccacc

SEQ ID NO: 52 - DNA, 50 bp, Homo sapiens
  misc_feature 1..50: note = synthetic read with codons 41/42 wildtype sequence
  source 1..50: mol_type = other DNA
gagtttcttggagacccaggttcccatctggtggtcgtcggattcccacc